European Patent Specification EP 3 413 922 B1, published December 10, 2025. Title: Improved sulfamide linkers for use in bioconjugates. Applicant: SynAffix B.V. The sequence listing filed with the application follows.

SEQUENCE LISTING (2 sequences)

SEQ ID NO: 1 - protein, 1258 aa, Artificial sequence
  Fusion protein EndoSH
MPSIDSLHYLSENSKKEFKEELSKAGQESQKVKEILAKAQQADKQAQELAKMKIPEKIPMKPLHGPLYGGYFRTWHDKTSDPTEKDKVNSMGELPKEVDLAFIFHDWTKDYSLFWKELATKHVPKLNKQGTRVIRTIPWRFLAGGDNSGIAEDTSKYPNTPEGNKALAKAIVDEYVYKYNLDGLDVDVEHDSIPKVDKKEDTAGVERSIQVFEEIGKLIGPKGVDKSRLFIMDSTYMADKNPLIERGAPYINLLLVQVYGSQGEKGGWEPVSNRPEKTMEERWQGYSKYIRPEQYMIGFSFYEENAQEGNLWYDINSRKDEDKANGINTDITGTRAERYARWQPKTGGVKGGIFSYAIDRDGVAHQPKKYAKQKEFKDATDNIFHSDYSVSKALKTVMLKDKSYDLIDEKDFPDKALREAVMAQVGTRKGDLERFNGTLRLDNPAIQSLEGLNKFKKLAQLDLIGLSRITKLDRSVLPANMKPGKDTLETVLETYKKDNKEEPATIPPVSLKVSGLTGLKELDLSGFDRETLAGLDAATLTSLEKVDISGNKLDLAPGTENRQIFDTMLSTISNHVGSNEQTVKFDKQKPTGHYPDTYGKTSLRLPVANEKVDLQSQLLFGTVTNQGTLINSEADYKAYQNHKIAGRSFVDSNYHYNNFKVSYENYTVKVTDSTLGTTTDKTLATDKEETYKVDFFSPADKTKAVHTAKVIVGDEKTMMVNLAEGATVIGGSADPVNARKVFDGQLGSETDNISLGWDSKQSIIFKLKEDGLIKHWRFFNDSARNPETTNKPIQEASLQIFNIKDYNLDNLLENPNKFDDEKYWITVDTYSAQGERATAFSNTLNNITSKYWRVVFDTKGDRYSSPVVPELQILGYPLPNADTIMKTVTTAKELSQQKDKFSQKMLDELKIKEMALETSLNSKIFDVTAINANAGVLKDCIEKRQLLKKGGGGSGGGGSGGGGSHHHHHHEFGGGGSGGGGSGGGGSAPAPVKQGPTSVAYVEVNNNSMLNVGKYTLADGGGNAFDVAVIFAANINYDTGTKTAYLHFNENVQRVLDNAVTQIRPLQQQGIKVLLSVLGNHQGAGFANFPSQQAASAFAKQLSDAVAKYGLDGVDFDDEYAEYGNNGTAQPNDSSFVHLVTALRANMPDKIISLYNIGPAASRLSYGGVDVSDKFDYAWNPYYGTWQVPGIALPKAQLSPAAVEIGRTSRSTVADLARRTVDEGYGVYLTYNLDGGDRTADVSAFTRELYGSEAVRTP

SEQ ID NO: 2 - protein, 410 aa, Artificial sequence
  His-TnGalNAcT(33-421)
MGSSHHHHHHSSGLVPRGSHMSPLRTYLYTPLYNATQPTLRNVERLAANWPKKIPSNYIEDSEEYSIKNISLSNHTTRASVVHPPSSITETASKLDKNMTIQDGAFAMISPTPLLITKLMDSIKSYVTTEDGVKKAEAVVTLPLCDSMPPDLGPITLNKTELELEWVEKKFPEVEWGGRYSPPNCTARHRVAIIVPYRDRQQHLAIFLNHMHPFLMKQQIEYGIFIVEQEGNKDFNRAKLMNVGFVESQKLVAEGWQCFVFHDIDLLPLDTRNLYSCPRQPRHMSASIDKLHFKLPYEDIFGGVSAMTLEQFTRVNGFSNKYWGWGGEDDDMSYRLKKINYHIARYKMSIARYAMLDHKKSTPNPKRYQLLSQTSKTFQKDGLSTLEYELVQVVQYHLYTHILVNIDERS